European Patent Application EP 4 389 884 A1, published June 26, 2024. Title: EFFICIENT PRODUCTION OF ENANTIOPURE D-3-HYDROXYBUTYRATE. Applicant: Helmut Schwab. The sequence listing filed with the application follows.

SEQUENCE LISTING (16 sequences)

SEQ ID NO: 1 - protein, 494 aa, Acidovorax sp.
MAFNFIRAAAAGAAMALCGAGGVHAAVNLPALKIDKTQTTVSGLSSGGFMAVQLHVAYSATFAKGAGVVAGGPFYCAEGSIVNATGRCMASPAGIPTSTLVSTTNTWASQGVIDPVANLQTSKVYLFSGTLDSVVKTGVMDALRTYYNSFVPAANVVYKKDIAAEHAMVTDDYGNACSTKGAPYISDCNFDLAGAMLQHLYGTLNARNNATLPTGNYIEFNQSEFITNHGMATTGWAYVPQACQAGGTATCKLHVVLHGCKQNISDVQQQYVRNTGYNRWADTNNIVMLYPQTSTAATNSCWDWWGYDSANYSKKSGPQMAAIKAMVDRVSSGTGGTTPPDPVALPAPTGVSTSGATASSMAIGWAAVTGAASYNVYRNANKVNALPVTATSYTDTGLAASTTYSWTVRAADANGAEGATSAAASGTTLAASGGGTATCTTASNYAHTLAGRAYAAGGYTYALGSNQNMGLWNVFVTNTLKQTSTNYYVIGTCP

SEQ ID NO: 2 - protein, 469 aa, Acidovorax sp.
AVNLPALKIDKTQTTVSGLSSGGFMAVQLHVAYSATFAKGAGVVAGGPFYCAEGSIVNATGRCMASPAGIPTSTLVSTTNTWASQGVIDPVANLQTSKVYLFSGTLDSVVKTGVMDALRTYYNSFVPAANVVYKKDIAAEHAMVTDDYGNACSTKGAPYISDCNFDLAGAMLQHLYGTLNARNNATLPTGNYIEFNQSEFITNHGMATTGWAYVPQACQAGGTATCKLHVVLHGCKQNISDVQQQYVRNTGYNRWADTNNIVMLYPQTSTAATNSCWDWWGYDSANYSKKSGPQMAAIKAMVDRVSSGTGGTTPPDPVALPAPTGVSTSGATASSMAIGWAAVTGAASYNVYRNANKVNALPVTATSYTDTGLAASTTYSWTVRAADANGAEGATSAAASGTTLAASGGGTATCTTASNYAHTLAGRAYAAGGYTYALGSNQNMGLWNVFVTNTLKQTSTNYYVIGTCP

SEQ ID NO: 3 - protein, 507 aa, synthetic construct
  source 1..507: note = polyhydroxybutyrate depolymerase as SEQ ID No. 1 comprising a C-terminal His-tag
MAFNFIRAAAAGAAMALCGAGGVHAAVNLPALKIDKTQTTVSGLSSGGFMAVQLHVAYSATFAKGAGVVAGGPFYCAEGSIVNATGRCMASPAGIPTSTLVSTTNTWASQGVIDPVANLQTSKVYLFSGTLDSVVKTGVMDALRTYYNSFVPAANVVYKKDIAAEHAMVTDDYGNACSTKGAPYISDCNFDLAGAMLQHLYGTLNARNNATLPTGNYIEFNQSEFITNHGMATTGWAYVPQACQAGGTATCKLHVVLHGCKQNISDVQQQYVRNTGYNRWADTNNIVMLYPQTSTAATNSCWDWWGYDSANYSKKSGPQMAAIKAMVDRVSSGTGGTTPPDPVALPAPTGVSTSGATASSMAIGWAAVTGAASYNVYRNANKVNALPVTATSYTDTGLAASTTYSWTVRAADANGAEGATSAAASGTTLAASGGGTATCTTASNYAHTLAGRAYAAGGYTYALGSNQNMGLWNVFVTNTLKQTSTNYYVIGTCPKLAAALEHHHHHH

SEQ ID NO: 4 - protein, 483 aa, synthetic construct
  source 1..483: note = polyhydroxybutyrate depolymerase as SEQ ID No. 3 without signal sequence
MAVNLPALKIDKTQTTVSGLSSGGFMAVQLHVAYSATFAKGAGVVAGGPFYCAEGSIVNATGRCMASPAGIPTSTLVSTTNTWASQGVIDPVANLQTSKVYLFSGTLDSVVKTGVMDALRTYYNSFVPAANVVYKKDIAAEHAMVTDDYGNACSTKGAPYISDCNFDLAGAMLQHLYGTLNARNNATLPTGNYIEFNQSEFITNHGMATTGWAYVPQACQAGGTATCKLHVVLHGCKQNISDVQQQYVRNTGYNRWADTNNIVMLYPQTSTAATNSCWDWWGYDSANYSKKSGPQMAAIKAMVDRVSSGTGGTTPPDPVALPAPTGVSTSGATASSMAIGWAAVTGAASYNVYRNANKVNALPVTATSYTDTGLAASTTYSWTVRAADANGAEGATSAAASGTTLAASGGGTATCTTASNYAHTLAGRAYAAGGYTYALGSNQNMGLWNVFVTNTLKQTSTNYYVIGTCPKLAAALEHHHHHH

SEQ ID NO: 5 - protein, 10 aa, synthetic construct
  source 1..10: note = enzyme motif
  VARIANT 5: note = X is threonine, serine, glycine, glutamic acid, glutamine or aspartic acid
ANLQXSKVYL

SEQ ID NO: 6 - protein, 19 aa, synthetic construct
  source 1..19: note = enzyme motif
  VARIANT 10: note = X is threonine, serine, glycine, glutamic acid, glutamine or aspartic acid
VIDPVANLQXSKVYLFSGT

SEQ ID NO: 7 - protein, 30 aa, synthetic construct
  source 1..30: note = enzyme motif
  VARIANT 11: note = X is threonine, serine, glycine, glutamic acid, glutamine or aspartic acid
GVIDPVANLQXSKVYLFSGTLDSVVKTGVM

SEQ ID NO: 8 - protein, 41 aa, synthetic construct
  source 1..41: note = enzyme motif
  VARIANT 12: note = X is threonine, serine, glycine, glutamic acid, glutamine or aspartic acid
QGVIDPVANLQXSKVYLFSGTLDSVVKTGVMDALRTYYNSF

SEQ ID NO: 9 - protein, 54 aa, synthetic construct
  source 1..54: note = enzyme motif
  VARIANT 12: note = X is threonine, serine, glycine, glutamic acid, glutamine or aspartic acid
QGVIDPVANLQXSKVYLFSGTLDSVVKTGVMDALRTYYNSFVPAANVVYKKDIA

SEQ ID NO: 10 - protein, 10 aa, synthetic construct
  source 1..10: note = enzyme motif
ANLQNSKVYL

SEQ ID NO: 11 - protein, 19 aa, synthetic construct
  source 1..19: note = enzyme motif
VIDPVANLQNSKVYLFSGT

SEQ ID NO: 12 - protein, 30 aa, synthetic construct
  source 1..30: note = enzyme motif
GVIDPVANLQNSKVYLFSGTLDSVVKTGVM

SEQ ID NO: 13 - protein, 41 aa, synthetic construct
  source 1..41: note = enzyme motif
QGVIDPVANLQNSKVYLFSGTLDSVVKTGVMDALRTYYNSF

SEQ ID NO: 14 - protein, 54 aa, synthetic construct
  source 1..54: note = enzyme motif
QGVIDPVANLQNSKVYLFSGTLDSVVKTGVMDALRTYYNSFVPAANVVYKKDIA

SEQ ID NO: 15 - protein, 10 aa, synthetic construct
  source 1..10: note = enzyme motif
GATANSMAIG

SEQ ID NO: 16 - protein, 12 aa, synthetic construct
  source 1..12: note = enzyme motif
SGATANSMAIGW